European Patent Application EP 4 155 323 A1, published March 29, 2023. Title: Novel Compositions and Methods for Treating IgE-Mediated Disorders. Applicant: Xencor, Inc. Desjarlais, John R. Chu, Seung Y Horton, Holly M. Application PCT/US2009/057366. The sequence listing filed with the application follows.

SEQUENCE LISTING (45 sequences)

SEQ ID NO: 1 - protein, 121 aa, Artificial Sequence [sequence omitted]

SEQ ID NO: 2 - protein, 9 aa, Mus musculus
YSITSGYSW

SEQ ID NO: 3 - protein, 5 aa, Mus musculus
TYDGS

SEQ ID NO: 4 - protein, 12 aa, Mus musculus
GSHYFGHWHFAV

SEQ ID NO: 5 - protein, 111 aa, Artificial Sequence [sequence omitted]

SEQ ID NO: 6 - protein, 10 aa, Mus musculus
QSVDYDGDSY

SEQ ID NO: 7 - protein, 7 aa, Mus musculus
AASYLES

SEQ ID NO: 8 - protein, 7 aa, Mus musculus
SHEDPYT

SEQ ID NO: 9 - protein, 121 aa, Mus musculus
DVQLQESGPGLVKPSQSLSLACSVTGYSITSGYSWNWIRQFPGNKLEWMGSITYDGSSNYNPSLKNRISVTRDTSQNQFFLKLNSATAEDTATYYCARGSHYFGHWHFAVWGAGTTVTVSS

SEQ ID NO: 10 - protein, 9 aa, Mus musculus
YSITSGYSW

SEQ ID NO: 11 - protein, 5 aa, Mus musculus
TYDGS

SEQ ID NO: 12 - protein, 12 aa, Mus musculus
GSHYFGHWHFAV

SEQ ID NO: 13 - protein, 111 aa, Mus musculus
DIQLTQSPASLAVSLGQRATISCKASQSVDYDGDSYMNWYQQKPGQPPILLIYAASYLGSEIPARFSGSGSGTDFTLNIHPVEEEDAATFYCQQSHEDPYTFGAGTKLEIK

SEQ ID NO: 14 - protein, 10 aa, Mus musculus
QSVDYDGDSY

SEQ ID NO: 15 - protein, 7 aa, Mus musculus
AASYLGS

SEQ ID NO: 16 - protein, 7 aa, Mus musculus
SHEDPYT

SEQ ID NO: 17 - protein, 121 aa, Artificial Sequence
  H1L1MaE11 VH Humanized
QVQLQESGPGLVKPSETLSLTCAVSGYSITSGYSWNWIRQPPGKKLEWIGSITYDGSSNYNPSLKSRVTISRDTSKNQFSLKLSSVTAADTAVYYCARGSHYFGHWHFAVWGAGTLVTVSS

SEQ ID NO: 18 - protein, 9 aa, Mus musculus
YSITSGYSW

SEQ ID NO: 19 - protein, 5 aa, Mus musculus
TYDGS

SEQ ID NO: 20 - protein, 12 aa, Mus musculus
GSHYFGHWHFAV

SEQ ID NO: 21 - protein, 111 aa, Mus musculus
DIQLTQSPSSLSASVGDRVTITCRASQSVDYDGDSYMNWYQQKPGQPPKLLIYAASYLGSEIPARFSGSGSGTDFTLTISSLQPEDFATYYCQQSHEDPYTFGAGTKLEIK

SEQ ID NO: 22 - protein, 10 aa, Mus musculus
QSVDYDGDSY

SEQ ID NO: 23 - protein, 7 aa, Mus musculus
AASYLGS

SEQ ID NO: 24 - protein, 7 aa, Mus musculus
SHEDPYT

SEQ ID NO: 25 - protein, 123 aa, Mus musculus
QVQLQQSGAELMKPGASVKISCKTTGYTFSMYWLEWVKQRPGHGLEWVGEISPGTFTTNYNEKFKAKATFTADTSSNTAYLQLSGLTSEDSAVYFCARFSHFSGSNYDYFDYWGQGTSLTVSS

SEQ ID NO: 26 - protein, 7 aa, Mus musculus
YTFSMYW

SEQ ID NO: 27 - protein, 6 aa, Mus musculus
SPGTFT

SEQ ID NO: 28 - protein, 14 aa, Mus musculus
FSHFSGSNYDYFDY

SEQ ID NO: 29 - protein, 107 aa, Mus musculus
DILLTQSPAILSVSPGERVSFSCRASQSIGTNIHWYQQRTDGSPRLLIKYASESISGIPSRFSGSGSGTEFTLNINSVESEDIADYYCQQSDSWPTTFGGGTKLEIK

SEQ ID NO: 30 - protein, 6 aa, Mus musculus
QSIGTN

SEQ ID NO: 31 - protein, 7 aa, Mus musculus
YASESIS

SEQ ID NO: 32 - protein, 7 aa, Mus musculus
SDSWPTT

SEQ ID NO: 33 - protein, 107 aa, Mus musculus [sequence omitted]

SEQ ID NO: 34 - protein, 330 aa, Mus musculus
ASTKGPSVFPLAPSSKSTSGGTAALGCLVKDYFPEPVTVSWNSGALTSGVHTFPAVLQSSGLYSLSSVVTVPSSSLGTQTYICNVNHKPSNTKVDKKVEPKSCDKTHTCPPCPAPELLGGPSVFLFPPKPKDTLMISRTPEVTCVVVDVSHEDPEVKFNWYVDGVEVHNAKTKPREEQYNSTYRVVSVLTVLHQDWLNGKEYKCKVSNKALPAPIEKTISKAKGQPREPQVYTLPPSREEMTKNQVSLTCLVKGFYPSDIAVEWESNGQPENNYKTTPPVLDSDGSFFLYSKLTVDKSRWQQGNVFSCSVMHEALHNHYTQKSLSLSPGK

SEQ ID NO: 35 - protein, 330 aa, Artificial Sequence
  S267E/L328F IgG1 constant chain Artificial Variant
ASTKGPSVFPLAPSSKSTSGGTAALGCLVKDYFPEPVTVSWNSGALTSGVHTFPAVLQSSGLYSLSSVVTVPSSSLGTQTYICNVNHKPSNTKVDKKVEPKSCDKTHTCPPCPAPELLGGPSVFLFPPKPKDTLMISRTPEVTCVVVDVEHEDPEVKFNWYVDGVEVHNAKTKPREEQYNSTYRVVSVLTVLHQDWLNGKEYKCKVSNKAFPAPIEKTISKAKGQPREPQVYTLPPSREEMTKNQVSLTCLVKGFYPSDIAVEWESNGQPENNYKTTPPVLDSDGSFFLYSKLTVDKSRWQQGNVFSCSVMHEALHNHYTQKSLSLSPGK

SEQ ID NO: 36 - protein, 330 aa, Artificial Sequence
  G236D/S267E IgG1 constant chain Artificial Variant
ASTKGPSVFPLAPSSKSTSGGTAALGCLVKDYFPEPVTVSWNSGALTSGVHTFPAVLQSSGLYSLSSVVTVPSSSLGTQTYICNVNHKPSNTKVDKKVEPKSCDKTHTCPPCPAPELLDGPSVFLFPPKPKDTLMISRTPEVTCVVVDVEHEDPEVKFNWYVDGVEVHNAKTKPREEQYNSTYRVVSVLTVLHQDWLNGKEYKCKVSNKALPAPIEKTISKAKGQPREPQVYTLPPSREEMTKNQVSLTCLVKGFYPSDIAVEWESNGQPENNYKTTPPVLDSDGSFFLYSKLTVDKSRWQQGNVFSCSVMHEALHNHYTQKSLSLSPGK

SEQ ID NO: 37 - protein, 218 aa, Artificial Sequence
  Omalizumab light chain (VH-C ) Artificial Variant
DIQLTQSPSSLSASVGDRVTITCRASQSVDYDGDSYMNWYQQKPGKAPKLLIYAASYLESGVPSRFSGSGSGTDFTLTISSLQPEDFATYYCQQSHEDPYTFGQGTKVEIKRTVAAPSVFIFPPSDEQLKSGTASVVCLLNNFYPREAKVQWKVDNALQSGNSQESVTEQDSKDSTYSLSSTLTLSKADYEKHKVYACEVTHQGLSSPVTKSFNRGEC

SEQ ID NO: 38 - protein, 451 aa, Artificial Sequence
  Omalizumab IgG1 heavy chain Artificial Variant
EVQLVESGGGLVQPGGSLRLSCAVSGYSITSGYSWNWIRQAPGKGLEWVASITYDGSTNYNPSVKGRITISRDDSKNTFYLQMNSLRAEDTAVYYCARGSHYFGHWHFAVWGQGTLVTVSSASTKGPSVFPLAPSSKSTSGGTAALGCLVKDYFPEPVTVSWNSGALTSGVHTFPAVLQSSGLYSLSSVVTVPSSSLGTQTYICNVNHKPSNTKVDKKVEPKSCDKTHTCPPCPAPELLGGPSVFLFPPKPKDTLMISRTPEVTCVVVDVSHEDPEVKFNWYVDGVEVHNAKTKPREEQYNSTYRVVSVLTVLHQDWLNGKEYKCKVSNKALPAPIEKTISKAKGQPREPQVYTLPPSREEMTKNQVSLTCLVKGFYPSDIAVEWESNGQPENNYKTTPPVLDSDGSFFLYSKLTVDKSRWQQGNVFSCSVMHEALHNHYTQKSLSLSPGK

SEQ ID NO: 39 - protein, 451 aa, Artificial Sequence
  Omalizumab S267E/L328F heavy chain Artificial Humanized
EVQLVESGGGLVQPGGSLRLSCAVSGYSITSGYSWNWIRQAPGKGLEWVASITYDGSTNYNPSVKGRITISRDDSKNTFYLQMNSLRAEDTAVYYCARGSHYFGHWHFAVWGQGTLVTVSSASTKGPSVFPLAPSSKSTSGGTAALGCLVKDYFPEPVTVSWNSGALTSGVHTFPAVLQSSGLYSLSSVVTVPSSSLGTQTYICNVNHKPSNTKVDKKVEPKSCDKTHTCPPCPAPELLGGPSVFLFPPKPKDTLMISRTPEVTCVVVDVEHEDPEVKFNWYVDGVEVHNAKTKPREEQYNSTYRVVSVLTVLHQDWLNGKEYKCKVSNKAFPAPIEKTISKAKGQPREPQVYTLPPSREEMTKNQVSLTCLVKGFYPSDIAVEWESNGQPENNYKTTPPVLDSDGSFFLYSKLTVDKSRWQQGNVFSCSVMHEALHNHYTQKSLSLSPGK

SEQ ID NO: 40 - protein, 218 aa, Artificial Sequence
  H1L1 MaE11 light chain (VH-C ) Artificial Humanized
DIQLTQSPSSLSASVGDRVTITCRASQSVDYDGDSYMNWYQQKPGQPPKLLIYAASYLGSEIPARFSGSGSGTDFTLTISSLQPEDFATYYCQQSHEDPYTFGAGTKLEIKRTVAAPSVFIFPPSDEQLKSGTASVVCLLNNFYPREAKVQWKVDNALQSGNSQESVTEQDSKDSTYSLSSTLTLSKADYEKHKVYACEVTHQGLSSPVTKSFNRGEC

SEQ ID NO: 41 - protein, 451 aa, Artificial Sequence
  H1L1 MaE11 IgG1 heavy chain Artificial Humanized
QVQLQESGPGLVKPSETLSLTCAVSGYSITSGYSWNWIRQPPGKKLEWIGSITYDGSSNYNPSLKSRVTISRDTSKNQFSLKLSSVTAADTAVYYCARGSHYFGHWHFAVWGAGTLVTVSSASTKGPSVFPLAPSSKSTSGGTAALGCLVKDYFPEPVTVSWNSGALTSGVHTFPAVLQSSGLYSLSSVVTVPSSSLGTQTYICNVNHKPSNTKVDKKVEPKSCDKTHTCPPCPAPELLGGPSVFLFPPKPKDTLMISRTPEVTCVVVDVSHEDPEVKFNWYVDGVEVHNAKTKPREEQYNSTYRVVSVLTVLHQDWLNGKEYKCKVSNKALPAPIEKTISKAKGQPREPQVYTLPPSREEMTKNQVSLTCLVKGFYPSDIAVEWESNGQPENNYKTTPPVLDSDGSFFLYSKLTVDKSRWQQGNVFSCSVMHEALHNHYTQKSLSLSPGK

SEQ ID NO: 42 - protein, 451 aa, Artificial Sequence
  H1L1 MaE11 S267E/L328F heavy chain Artificial Humanized
QVQLQESGPGLVKPSETLSLTCAVSGYSITSGYSWNWIRQPPGKKLEWIGSITYDGSSNYNPSLKSRVTISRDTSKNQFSLKLSSVTAADTAVYYCARGSHYFGHWHFAVWGAGTLVTVSSASTKGPSVFPLAPSSKSTSGGTAALGCLVKDYFPEPVTVSWNSGALTSGVHTFPAVLQSSGLYSLSSVVTVPSSSLGTQTYICNVNHKPSNTKVDKKVEPKSCDKTHTCPPCPAPELLGGPSVFLFPPKPKDTLMISRTPEVTCVVVDVEHEDPEVKFNWYVDGVEVHNAKTKPREEQYNSTYRVVSVLTVLHQDWLNGKEYKCKVSNKAFPAPIEKTISKAKGQPREPQVYTLPPSREEMTKNQVSLTCLVKGFYPSDIAVEWESNGQPENNYKTTPPVLDSDGSFFLYSKLTVDKSRWQQGNVFSCSVMHEALHNHYTQKSLSLSPGK

SEQ ID NO: 43 - DNA, 5 bp, Artificial Sequence
  glycine-serine linker
gsggs

SEQ ID NO: 44 - DNA, 5 bp, Artificial Sequence
  glycine-serine linker
ggggs

SEQ ID NO: 45 - DNA, 4 bp, Artificial Sequence
  glycine-serine linker
gggs